European Patent Application EP 4 686 726 A1, published February 4, 2026. Title: MICROBIAL PRODUCTION OF RECOMBINANT MINK HAIR KERATINS FOR TEXTILE APPLICATIONS. Applicant: Fendi SRL. The sequence listing filed with the application follows.

SEQUENCE LISTING (44 sequences)

SEQ ID NO: 1 - protein, 409 aa, Neogale vison
MPYNCCLPNVSCRSTCSSRPCVPPSCHTCTLPGACNIPANVGNCGWFCEGSFNGSEKETMQFLNDRLASYLEKVRQLERENAELESRIRERCQQQEPYVCPSYQSYFRTIEELQQKILCAKSENARLVVQIDNAKLAADDFRTKYETELGLRQLVESDINGLRRILDELTLCKSDLEAQVESLKEELLCLKRNHEEEVNTLRCQIGDRLNVEVDAAPAVDLNRVLNETRCQYEALVETNRRDVEEWFTTQTEELNKQVVSSSEQLQSCQAEIIELRRTVNALEIELQAQHNLRDSLENTLTETEARYSSQLSQLQCMITNVESQLAEIRSDLERQNQEYQVLLDVRARLECEINTYRGLLESEDCKLPCNPCATTNACGSSGSCVSNSCAPCTPCVPRPRCGPCNSFVR

SEQ ID NO: 2 - protein, 455 aa, Neogale vison
MASKCLKASFSSGSLRGLGGAGGGSARVSAIYPSSSCKLPSLSRGARSFSACSVGLGRSSSRAAGCLSALCLPAGGFTTSYNLGGGWFGDGILTGSEKETMQSLNDRLASYLEKVRQLERENASLEGRIREWCEQQVPYLSPDYQSYFRTIEELQKKTLCTKAENARLVVQIDNAKLAADDFRTKYETELSMRQLVESDMNGLRRILDDLTLCKSDLEAQVESLKEELLCLKKNHEEEVNSLRCQLGDRLNVEVDAAPPVDLNRVLDEMRCQYETLVENNRRDAEEWFNTQTEELNQQVVSSSEQLQSCQAEIIELRRSVNALEIELQAQQSMRDALESTLAETEARYSSQLAQMQCLISNVEAQLAEIRSDLERQNQEYQVLLDVRARLECEINTYRGLLESEEGKLPCNPCAPDHTPGKSCLPCLPAVSCGPGAVRSTCSPRTICVPCPGGRF

SEQ ID NO: 3 - protein, 519 aa, Neogale vison
MTCGSGFCGRAFSCISACGPRPGRCCITAAPYRGVSCYRGLTGGFGSHSVCGGFRAGSCGRSFGYRSGGVCGPSPPCITSVSVNESLLTPLNLEIDPNAQCVKHEEKEQIKCLNSRFAAFIDKVRFLEQQNKLLETKWQFYQNRKCCESNLEPLFEGYIETLRREAECVEADSGRLASELNHVQEVLEGYKKKYEEEVALRATAENEFVALKKDVDCAYLRKSDLEANAEALTEEIDFLRRLYEEEIRVLHAHISDTSVIVKMDNSRDLNMDCIVAEIKAQYDDIASRSRAEAESWYRSKCEEMKATVIRHGETLRRTKEEINELNRMIQRLTAEVENAKCQNTKLEAAVTQAEQQGETALSDARCKLAELEAALQKAKQDMACLVKEYQEVMNSKLGLDIEIATYRRLLEGEEQRLCEGVGAVNVCVSSSRGGVVCGDLCVSGSRPVTGSACSAPCSGNLAVSTGMCAPCAPCAPCAPCAPCGPCNSVTSCGLGTGGVGSCGISSCGVGSCASSCRRC

SEQ ID NO: 4 - protein, 507 aa, Neogale vison
MSCRSYRISSGCGVTRTFSSCSAVAPKTGNRCCISAAPYRGVSCYRGLTGFGSRSLSNLGSCGPRMAMGGFRAGSCGRSFGYRSGGVCGPSPPCITTVSVNESLLTPLNLEIDPNAQCVKHEEKEQIKCLNNRFAAFIDKVRFLEQQNKLLETKWQFYQNQRCCESNMEPLFNGYIETLRREAECVEADSGRLASELNHVQEVLEGYKKKYEEEVALRATAENEFVVLKKDVDCAYLRKSDLEANVEALVEESSFLKRLYDEELQVLHAHISDTSVIVKMDNSRDLNMDCVVAEIKAQYDDIASRSRAEAESWYRSKCEEMKATVIRHGETLRRTKEEINELNRMIQRLTAEIENAKCQRAKLEAAVAEAEQQGEAALTDARCKLAELEAALQKAKQDMACLLKEYQEVMNSKLGLDIEIATYRRLLEGEEHRLCEGVGSVNVCVSSSRGGVACGGLTCSTTPGRQIASGPVATGGSITVMAPDSCAPCQPRSSSFSCGSSRSVRFA

SEQ ID NO: 5 - protein, 442 aa, Neogale vison
MTSNCSASIKSCPRPSSVCSSSMSCRPEMCLGYVCQPVSCVPSVSMPTTYRPASCFSKTYLSSSCWAASGISSSMGTCSWFCEGSFNGNEKETMQSLNDRLACYLEKVRQLERENAELESKIQEACQSQVATMSPDYQSYFRTIEELQQKVLCTKAENARMVVHIDNAKLAADDFRTKYETELTMRQLVEADTNGLRRILDELTLCKADLEAQVESLKEELLCLKKNHEQEVSALRCQLGDRLNIEVDAAPPVDLNRMLEEMRCQYETVVEANLRDVEEWFNTQMEELNQQVATSSEQLQSYQSDIIDLRRTVNTLEIELQAQHSLRDSLESTLAETEARYGSQLAQMQCLISNVEAQLAEIRCDLERQNQEYKVLLDVKARLECEINTYRGLLESEDCKLPCNPCSTPSCPPCAPSPSMPRTVCVPRTVCVPCVPCPQSRF

SEQ ID NO: 6 - protein, 510 aa, Neogale vison
MSCRSFQLGSRCGGRSFSSCSAVLPRMVTHYAVSKGPCQSGGGSALRALGCLGSRSLCNVGFGRPRVASRCGLPGFGYRVGAPCGSSPCIAPVTINESLLVPLELEIDPAVQKVKRDEKEQIKCLNNRFASFINKVRFLEQKNKLLETKWNFMQQQRCCQSNIEPIFQAYISALRRQLDCVAGDRARLESELCSLQDVLESYKKKYEEELSLRPCAENEFVALKKDVDTAFLMKADLETNAEALVQEIDFLKGLYEEEICLLQSQISETSVIVKMDNSRELDVDGIIAEIKAQYDDIASRSKAEAEAWYQSRYEELRLTAGNHCDNLRNRKNEILEMNKLIQRLQQEIENVKAQRCKLEAAVTQAEQQGEAALSDAKCKLVGLEEALQKAKQDMACLLKEYQEVMNSKLGLDIEIATYRRLLEGEEHRLCEGIGPVNISVSSSKGAVLYEPCVVSTPVLRTGVLKTSGACSVVGTGEVYVPCEPQGLLSCVSTRSSCMKLGAGSSSSHKC

SEQ ID NO: 7 - protein, 443 aa, synthetic construct
  source 1..443: note = His-KRT31 fusion protein
MGSSHHHHHHSSGLVPRGSHMASMTGGQQMGRDGMPYNCCLPNVSCRSTCSSRPCVPPSCHTCTLPGACNIPANVGNCGWFCEGSFNGSEKETMQFLNDRLASYLEKVRQLERENAELESRIRERCQQQEPYVCPSYQSYFRTIEELQQKILCAKSENARLVVQIDNAKLAADDFRTKYETELGLRQLVESDINGLRRILDELTLCKSDLEAQVESLKEELLCLKRNHEEEVNTLRCQIGDRLNVEVDAAPAVDLNRVLNETRCQYEALVETNRRDVEEWFTTQTEELNKQVVSSSEQLQSCQAEIIELRRTVNALEIELQAQHNLRDSLENTLTETEARYSSQLSQLQCMITNVESQLAEIRSDLERQNQEYQVLLDVRARLECEINTYRGLLESEDCKLPCNPCATTNACGSSGSCVSNSCAPCTPCVPRPRCGPCNSFVR

SEQ ID NO: 8 - protein, 489 aa, synthetic construct
  source 1..489: note = His-KRT35 fusion protein
MGSSHHHHHHSSGLVPRGSHMASMTGGQQMGRDGMASKCLKASFSSGSLRGLGGAGGGSARVSAIYPSSSCKLPSLSRGARSFSACSVGLGRSSSRAAGCLSALCLPAGGFTTSYNLGGGWFGDGILTGSEKETMQSLNDRLASYLEKVRQLERENASLEGRIREWCEQQVPYLSPDYQSYFRTIEELQKKTLCTKAENARLVVQIDNAKLAADDFRTKYETELSMRQLVESDMNGLRRILDDLTLCKSDLEAQVESLKEELLCLKKNHEEEVNSLRCQLGDRLNVEVDAAPPVDLNRVLDEMRCQYETLVENNRRDAEEWFNTQTEELNQQVVSSSEQLQSCQAEIIELRRSVNALEIELQAQQSMRDALESTLAETEARYSSQLAQMQCLISNVEAQLAEIRSDLERQNQEYQVLLDVRARLECEINTYRGLLESEEGKLPCNPCAPDHTPGKSCLPCLPAVSCGPGAVRSTCSPRTICVPCPGGRF

SEQ ID NO: 9 - protein, 553 aa, synthetic construct
  source 1..553: note = His-KRT81 fusion protein
MGSSHHHHHHSSGLVPRGSHMASMTGGQQMGRDGMTCGSGFCGRAFSCISACGPRPGRCCITAAPYRGVSCYRGLTGGFGSHSVCGGFRAGSCGRSFGYRSGGVCGPSPPCITSVSVNESLLTPLNLEIDPNAQCVKHEEKEQIKCLNSRFAAFIDKVRFLEQQNKLLETKWQFYQNRKCCESNLEPLFEGYIETLRREAECVEADSGRLASELNHVQEVLEGYKKKYEEEVALRATAENEFVALKKDVDCAYLRKSDLEANAEALTEEIDFLRRLYEEEIRVLHAHISDTSVIVKMDNSRDLNMDCIVAEIKAQYDDIASRSRAEAESWYRSKCEEMKATVIRHGETLRRTKEEINELNRMIQRLTAEVENAKCQNTKLEAAVTQAEQQGETALSDARCKLAELEAALQKAKQDMACLVKEYQEVMNSKLGLDIEIATYRRLLEGEEQRLCEGVGAVNVCVSSSRGGVVCGDLCVSGSRPVTGSACSAPCSGNLAVSTGMCAPCAPCAPCAPCAPCGPCNSVTSCGLGTGGVGSCGISSCGVGSCASSCRRC

SEQ ID NO: 10 - protein, 541 aa, synthetic construct
  source 1..541: note = His-KRT85 fusion protein
MGSSHHHHHHSSGLVPRGSHMASMTGGQQMGRDGMSCRSYRISSGCGVTRTFSSCSAVAPKTGNRCCISAAPYRGVSCYRGLTGFGSRSLSNLGSCGPRMAMGGFRAGSCGRSFGYRSGGVCGPSPPCITTVSVNESLLTPLNLEIDPNAQCVKHEEKEQIKCLNNRFAAFIDKVRFLEQQNKLLETKWQFYQNQRCCESNMEPLFNGYIETLRREAECVEADSGRLASELNHVQEVLEGYKKKYEEEVALRATAENEFVVLKKDVDCAYLRKSDLEANVEALVEESSFLKRLYDEELQVLHAHISDTSVIVKMDNSRDLNMDCVVAEIKAQYDDIASRSRAEAESWYRSKCEEMKATVIRHGETLRRTKEEINELNRMIQRLTAEIENAKCQRAKLEAAVAEAEQQGEAALTDARCKLAELEAALQKAKQDMACLLKEYQEVMNSKLGLDIEIATYRRLLEGEEHRLCEGVGSVNVCVSSSRGGVACGGLTCSTTPGRQIASGPVATGGSITVMAPDSCAPCQPRSSSFSCGSSRSVRFA

SEQ ID NO: 11 - protein, 476 aa, synthetic construct
  source 1..476: note = His-KRT32 fusion protein
MGSSHHHHHHSSGLVPRGSHMASMTGGQQMGRDGMTSNCSASIKSCPRPSSVCSSSMSCRPEMCLGYVCQPVSCVPSVSMPTTYRPASCFSKTYLSSSCWAASGISSSMGTCSWFCEGSFNGNEKETMQSLNDRLACYLEKVRQLERENAELESKIQEACQSQVATMSPDYQSYFRTIEELQQKVLCTKAENARMVVHIDNAKLAADDFRTKYETELTMRQLVEADTNGLRRILDELTLCKADLEAQVESLKEELLCLKKNHEQEVSALRCQLGDRLNIEVDAAPPVDLNRMLEEMRCQYETVVEANLRDVEEWFNTQMEELNQQVATSSEQLQSYQSDIIDLRRTVNTLEIELQAQHSLRDSLESTLAETEARYGSQLAQMQCLISNVEAQLAEIRCDLERQNQEYKVLLDVKARLECEINTYRGLLESEDCKLPCNPCSTPSCPPCAPSPSMPRTVCVPRTVCVPCVPCPQSRF

SEQ ID NO: 12 - protein, 544 aa, synthetic construct
  source 1..544: note = His-KRT82 fusion protein
MGSSHHHHHHSSGLVPRGSHMASMTGGQQMGRDGMSCRSFQLGSRCGGRSFSSCSAVLPRMVTHYAVSKGPCQSGGGSALRALGCLGSRSLCNVGFGRPRVASRCGLPGFGYRVGAPCGSSPCIAPVTINESLLVPLELEIDPAVQKVKRDEKEQIKCLNNRFASFINKVRFLEQKNKLLETKWNFMQQQRCCQSNIEPIFQAYISALRRQLDCVAGDRARLESELCSLQDVLESYKKKYEEELSLRPCAENEFVALKKDVDTAFLMKADLETNAEALVQEIDFLKGLYEEEICLLQSQISETSVIVKMDNSRELDVDGIIAEIKAQYDDIASRSKAEAEAWYQSRYEELRLTAGNHCDNLRNRKNEILEMNKLIQRLQQEIENVKAQRCKLEAAVTQAEQQGEAALSDAKCKLVGLEEALQKAKQDMACLLKEYQEVMNSKLGLDIEIATYRRLLEGEEHRLCEGIGPVNISVSSSKGAVLYEPCVVSTPVLRTGVLKTSGACSVVGTGEVYVPCEPQGLLSCVSTRSSCMKLGAGSSSSHKC

SEQ ID NO: 13 - protein, 87 aa, synthetic construct
  source 1..87: note = alpha factor signal peptide
MRFPSIFTAVLFAASSALAAPVNTTTEDETAQIPAEAVIGYLDLEGDFDVAVLPFSNSTNNGLLFINTTIASIAAKEEGVSLDKREA

SEQ ID NO: 14 - protein, 19 aa, synthetic construct
  source 1..19: note = Invertase 2 signal peptide
MLLQAFLFLLAGFAAKISA

SEQ ID NO: 15 - protein, 46 aa, synthetic construct
  source 1..46: note = Wild-type UPO signal peptide
MRGTPIFASLIALFAHAAIAFPAYGSLAGLTREQLDEILPTLEIRA

SEQ ID NO: 16 - protein, 26 aa, synthetic construct
  source 1..26: note = Killer protein signal peptide
MTKPTQVLVRSVSILFFITLLHLVVA

SEQ ID NO: 17 - protein, 19 aa, synthetic construct
  source 1..19: note = secretion signal of the Kph-0030 protein
MKFAISTLLILQAAAVFAA

SEQ ID NO: 18 - protein, 92 aa, synthetic construct
  source 1..92: note = genetic fusion of a pre-alpha sequence to Ost1 co-translocation signal
MRQVWFSWIVGLFLCFFNVSSAAPVNTTTEDETAQIPAEAVIGYSDLEGDFDVAVLPFSNSTNNGLLFINTTIASIAAKEEGVSLEKREAEA

SEQ ID NO: 19 - protein, 507 aa, synthetic construct
  source 1..507: note = preostalpha SP-KRT31 fusion protein
MRQVWFSWIVGLFLCFFNVSSAAPVNTTTEDETAQIPAEAVIGYSDLEGDFDVAVLPFSNSTNNGLLFINTTIASIAAKEEGVSLEKREAEAPYNFCLPSLSCRTSCSSRPCVPPSCHSCTLPGACNIPANVSNCNWFCEGSFNGSEKETMQFLNDRLASYLEKVRQLERDNAELENLIRERSQQQEPLLCPSYQSYFKTIEELQQKILCTKSENARLVVQIDNAKLAADDFRTKYQTELSLRQLVESDINGLRRILDELTLCKSDLEAQVESLKEELLCLKSNHEQEVNTLRCQLGDRLNVEVDAAPTVDLNRVLNETRSQYEALVETNRREVEQWFTTQTEELNKQVVSSSEQLQSYQAEIIELRRTVNALEIELQAQHNLRDSLENTLTESEARYSSQLSQVQSLITNVESQLAEIRSDLERQNQEYQVLLDVRARLECEINTYRSLLESEDCNLPSNPCATTNACSKPIGPCLSNPCTSCVPPAPCTPCAPRPRCGPCNSFVR

SEQ ID NO: 20 - protein, 495 aa, synthetic construct
  source 1..495: note = Sce prepo alpha SP-KRT31 fusion protein
MRFPSIFTAVLFAASSALAAPVNTTTEDETAQIPAEAVIGYLDLEGDFDVAVLPFSNSTNNGLLFINTTIASIAAKEEGVSLDKREAPYNCCLPNVSCRSTCSSRPCVPPSCHTCTLPGACNIPANVGNCGWFCEGSFNGSEKETMQFLNDRLASYLEKVRQLERENAELESRIRERCQQQEPYVCPSYQSYFRTIEELQQKILCAKSENARLVVQIDNAKLAADDFRTKYETELGLRQLVESDINGLRRILDELTLCKSDLEAQVESLKEELLCLKRNHEEEVNTLRCQIGDRLNVEVDAAPAVDLNRVLNETRCQYEALVETNRRDVEEWFTTQTEELNKQVVSSSEQLQSCQAEIIELRRTVNALEIELQAQHNLRDSLENTLTETEARYSSQLSQLQCMITNVESQLAEIRSDLERQNQEYQVLLDVRARLECEINTYRGLLESEDCKLPCNPCATTNACGSSGSCVSNSCAPCTPCVPRPRCGPCNSFVR

SEQ ID NO: 21 - protein, 487 aa, synthetic construct
  source 1..487: note = Gma UPO SP-KRT32 fusion protein
MRGTPIFASLIALFAHAAIAFPAYGSLAGLTREQLDEILPTLEIRATSNCSASIKSCPRPSSVCSSSMSCRPEMCLGYVCQPVSCVPSVSMPTTYRPASCFSKTYLSSSCWAASGISSSMGTCSWFCEGSFNGNEKETMQSLNDRLACYLEKVRQLERENAELESKIQEACQSQVATMSPDYQSYFRTIEELQQKVLCTKAENARMVVHIDNAKLAADDFRTKYETELTMRQLVEADTNGLRRILDELTLCKADLEAQVESLKEELLCLKKNHEQEVSALRCQLGDRLNIEVDAAPPVDLNRMLEEMRCQYETVVEANLRDVEEWFNTQMEELNQQVATSSEQLQSYQSDIIDLRRTVNTLEIELQAQHSLRDSLESTLAETEARYGSQLAQMQCLISNVEAQLAEIRCDLERQNQEYKVLLDVKARLECEINTYRGLLESEDCKLPCNPCSTPSCPPCAPSPSMPRTVCVPRTVCVPCVPCPQSRF

SEQ ID NO: 22 - protein, 601 aa, synthetic construct
  source 1..601: note = preostalpha SP-KRT82 fusion protein
MRQVWFSWIVGLFLCFFNVSSAAPVNTTTEDETAQIPAEAVIGYSDLEGDFDVAVLPFSNSTNNGLLFINTTIASIAAKEEGVSLEKREAEASCRSFQLGSRCGGRSFSSCSAVLPRMVTHYAVSKGPCQSGGGSALRALGCLGSRSLCNVGFGRPRVASRCGLPGFGYRVGAPCGSSPCIAPVTINESLLVPLELEIDPAVQKVKRDEKEQIKCLNNRFASFINKVRFLEQKNKLLETKWNFMQQQRCCQSNIEPIFQAYISALRRQLDCVAGDRARLESELCSLQDVLESYKKKYEEELSLRPCAENEFVALKKDVDTAFLMKADLETNAEALVQEIDFLKGLYEEEICLLQSQISETSVIVKMDNSRELDVDGIIAEIKAQYDDIASRSKAEAEAWYQSRYEELRLTAGNHCDNLRNRKNEILEMNKLIQRLQQEIENVKAQRCKLEAAVTQAEQQGEAALSDAKCKLVGLEEALQKAKQDMACLLKEYQEVMNSKLGLDIEIATYRRLLEGEEHRLCEGIGPVNISVSSSKGAVLYEPCVVSTPVLRTGVLKTSGACSVVGTGEVYVPCEPQGLLSCVSTRSSCMKLGAGSSSSHKC

SEQ ID NO: 23 - protein, 532 aa, synthetic construct
  source 1..532: note = Killer protein SP-KRT85 fusion protein
MTKPTQVLVRSVSILFFITLLHLVVASCRSYRISSGCGVTRTFSSCSAVAPKTGNRCCISAAPYRGVSCYRGLTGFGSRSLSNLGSCGPRMAMGGFRAGSCGRSFGYRSGGVCGPSPPCITTVSVNESLLTPLNLEIDPNAQCVKHEEKEQIKCLNNRFAAFIDKVRFLEQQNKLLETKWQFYQNQRCCESNMEPLFNGYIETLRREAECVEADSGRLASELNHVQEVLEGYKKKYEEEVALRATAENEFVVLKKDVDCAYLRKSDLEANVEALVEESSFLKRLYDEELQVLHAHISDTSVIVKMDNSRDLNMDCVVAEIKAQYDDIASRSRAEAESWYRSKCEEMKATVIRHGETLRRTKEEINELNRMIQRLTAEIENAKCQRAKLEAAVAEAEQQGEAALTDARCKLAELEAALQKAKQDMACLLKEYQEVMNSKLGLDIEIATYRRLLEGEEHRLCEGVGSVNVCVSSSRGGVACGGLTCSTTPGRQIASGPVATGGSITVMAPDSCAPCQPRSSSFSCGSSRSVRFA

SEQ ID NO: 24 - protein, 480 aa, synthetic construct
  source 1..480: note = Killer protein SP-KRT35 fusion protein
MTKPTQVLVRSVSILFFITLLHLVVAASKCLKASFSSGSLRGLGGAGGGSARVSAIYPSSSCKLPSLSRGARSFSACSVGLGRSSSRAAGCLSALCLPAGGFTTSYNLGGGWFGDGILTGSEKETMQSLNDRLASYLEKVRQLERENASLEGRIREWCEQQVPYLSPDYQSYFRTIEELQKKTLCTKAENARLVVQIDNAKLAADDFRTKYETELSMRQLVESDMNGLRRILDDLTLCKSDLEAQVESLKEELLCLKKNHEEEVNSLRCQLGDRLNVEVDAAPPVDLNRVLDEMRCQYETLVENNRRDAEEWFNTQTEELNQQVVSSSEQLQSCQAEIIELRRSVNALEIELQAQQSMRDALESTLAETEARYSSQLAQMQCLISNVEAQLAEIRSDLERQNQEYQVLLDVRARLECEINTYRGLLESEEGKLPCNPCAPDHTPGKSCLPCLPAVSCGPGAVRSTCSPRTICVPCPGGRF

SEQ ID NO: 25 - protein, 605 aa, synthetic construct
  source 1..605: note = alpha factor SP-KRT81 fusion protein
MRFPSIFTAVLFAASSALAAPVNTTTEDETAQIPAEAVIGYLDLEGDFDVAVLPFSNSTNNGLLFINTTIASIAAKEEGVSLDKREATCGSGFCGRAFSCISACGPRPGRCCITAAPYRGVSCYRGLTGGFGSHSVCGGFRAGSCGRSFGYRSGGVCGPSPPCITSVSVNESLLTPLNLEIDPNAQCVKHEEKEQIKCLNSRFAAFIDKVRFLEQQNKLLETKWQFYQNRKCCESNLEPLFEGYIETLRREAECVEADSGRLASELNHVQEVLEGYKKKYEEEVALRATAENEFVALKKDVDCAYLRKSDLEANAEALTEEIDFLRRLYEEEIRVLHAHISDTSVIVKMDNSRDLNMDCIVAEIKAQYDDIASRSRAEAESWYRSKCEEMKATVIRHGETLRRTKEEINELNRMIQRLTAEVENAKCQNTKLEAAVTQAEQQGETALSDARCKLAELEAALQKAKQDMACLVKEYQEVMNSKLGLDIEIATYRRLLEGEEQRLCEGVGAVNVCVSSSRGGVVCGDLCVSGSRPVTGSACSAPCSGNLAVSTGMCAPCAPCAPCAPCAPCGPCNSVTSCGLGTGGVGSCGISSCGVGSCASSCRRC

SEQ ID NO: 26 - protein, 427 aa, synthetic construct
  source 1..427: note = 0030 SP-KRT31 fusion protein
MKFAISTLLILQAAAVFAAPYNCCLPNVSCRSTCSSRPCVPPSCHTCTLPGACNIPANVGNCGWFCEGSFNGSEKETMQFLNDRLASYLEKVRQLERENAELESRIRERCQQQEPYVCPSYQSYFRTIEELQQKILCAKSENARLVVQIDNAKLAADDFRTKYETELGLRQLVESDINGLRRILDELTLCKSDLEAQVESLKEELLCLKRNHEEEVNTLRCQIGDRLNVEVDAAPAVDLNRVLNETRCQYEALVETNRRDVEEWFTTQTEELNKQVVSSSEQLQSCQAEIIELRRTVNALEIELQAQHNLRDSLENTLTETEARYSSQLSQLQCMITNVESQLAEIRSDLERQNQEYQVLLDVRARLECEINTYRGLLESEDCKLPCNPCATTNACGSSGSCVSNSCAPCTPCVPRPRCGPCNSFVR

SEQ ID NO: 27 - protein, 460 aa, synthetic construct
  source 1..460: note = 0030 SP-KRT32 fusion protein
MKFAISTLLILQAAAVFAATSNCSASIKSCPRPSSVCSSSMSCRPEMCLGYVCQPVSCVPSVSMPTTYRPASCFSKTYLSSSCWAASGISSSMGTCSWFCEGSFNGNEKETMQSLNDRLACYLEKVRQLERENAELESKIQEACQSQVATMSPDYQSYFRTIEELQQKVLCTKAENARMVVHIDNAKLAADDFRTKYETELTMRQLVEADTNGLRRILDELTLCKADLEAQVESLKEELLCLKKNHEQEVSALRCQLGDRLNIEVDAAPPVDLNRMLEEMRCQYETVVEANLRDVEEWFNTQMEELNQQVATSSEQLQSYQSDIIDLRRTVNTLEIELQAQHSLRDSLESTLAETEARYGSQLAQMQCLISNVEAQLAEIRCDLERQNQEYKVLLDVKARLECEINTYRGLLESEDCKLPCNPCSTPSCPPCAPSPSMPRTVCVPRTVCVPCVPCPQSRF

SEQ ID NO: 28 - protein, 528 aa, synthetic construct
  source 1..528: note = 0030 SP-KRT82 fusion protein
MKFAISTLLILQAAAVFAASCRSFQLGSRCGGRSFSSCSAVLPRMVTHYAVSKGPCQSGGGSALRALGCLGSRSLCNVGFGRPRVASRCGLPGFGYRVGAPCGSSPCIAPVTINESLLVPLELEIDPAVQKVKRDEKEQIKCLNNRFASFINKVRFLEQKNKLLETKWNFMQQQRCCQSNIEPIFQAYISALRRQLDCVAGDRARLESELCSLQDVLESYKKKYEEELSLRPCAENEFVALKKDVDTAFLMKADLETNAEALVQEIDFLKGLYEEEICLLQSQISETSVIVKMDNSRELDVDGIIAEIKAQYDDIASRSKAEAEAWYQSRYEELRLTAGNHCDNLRNRKNEILEMNKLIQRLQQEIENVKAQRCKLEAAVTQAEQQGEAALSDAKCKLVGLEEALQKAKQDMACLLKEYQEVMNSKLGLDIEIATYRRLLEGEEHRLCEGIGPVNISVSSSKGAVLYEPCVVSTPVLRTGVLKTSGACSVVGTGEVYVPCEPQGLLSCVSTRSSCMKLGAGSSSSHKC

SEQ ID NO: 29 - protein, 525 aa, synthetic construct
  source 1..525: note = Invertase 2 SP-KRT85 fusion protein
MLLQAFLFLLAGFAAKISASCRSYRISSGCGVTRTFSSCSAVAPKTGNRCCISAAPYRGVSCYRGLTGFGSRSLSNLGSCGPRMAMGGFRAGSCGRSFGYRSGGVCGPSPPCITTVSVNESLLTPLNLEIDPNAQCVKHEEKEQIKCLNNRFAAFIDKVRFLEQQNKLLETKWQFYQNQRCCESNMEPLFNGYIETLRREAECVEADSGRLASELNHVQEVLEGYKKKYEEEVALRATAENEFVVLKKDVDCAYLRKSDLEANVEALVEESSFLKRLYDEELQVLHAHISDTSVIVKMDNSRDLNMDCVVAEIKAQYDDIASRSRAEAESWYRSKCEEMKATVIRHGETLRRTKEEINELNRMIQRLTAEIENAKCQRAKLEAAVAEAEQQGEAALTDARCKLAELEAALQKAKQDMACLLKEYQEVMNSKLGLDIEIATYRRLLEGEEHRLCEGVGSVNVCVSSSRGGVACGGLTCSTTPGRQIASGPVATGGSITVMAPDSCAPCQPRSSSFSCGSSRSVRFA

SEQ ID NO: 30 - protein, 558 aa, synthetic construct
  source 1..558: note = preostalpha SP-KRT31-His2 fusion protein
MRQVWFSWIVGLFLCFFNVSSAAPVNTTTEDETAQIPAEAVIGYSDLEGDFDVAVLPFSNSTNNGLLFINTTIASIAAKEEGVSLEKREAEAPYNFCLPSLSCRTSCSSRPCVPPSCHSCTLPGACNIPANVSNCNWFCEGSFNGSEKETMQFLNDRLASYLEKVRQLERDNAELENLIRERSQQQEPLLCPSYQSYFKTIEELQQKILCTKSENARLVVQIDNAKLAADDFRTKYQTELSLRQLVESDINGLRRILDELTLCKSDLEAQVESLKEELLCLKSNHEQEVNTLRCQLGDRLNVEVDAAPTVDLNRVLNETRSQYEALVETNRREVEQWFTTQTEELNKQVVSSSEQLQSYQAEIIELRRTVNALEIELQAQHNLRDSLENTLTESEARYSSQLSQVQSLITNVESQLAEIRSDLERQNQEYQVLLDVRARLECEINTYRSLLESEDCNLPSNPCATTNACSKPIGPCLSNPCTSCVPPAPCTPCAPRPRCGPCNSFVRSGGSGGGHHHHHHGGSGGSHHHHHHDGGSGGGSTSRDHMVLHEYVNAAGIT

SEQ ID NO: 31 - protein, 546 aa, synthetic construct
  source 1..546: note = Sce prepro alpha SP-KRT31-His2 fusion protein
MRFPSIFTAVLFAASSALAAPVNTTTEDETAQIPAEAVIGYLDLEGDFDVAVLPFSNSTNNGLLFINTTIASIAAKEEGVSLDKREAPYNCCLPNVSCRSTCSSRPCVPPSCHTCTLPGACNIPANVGNCGWFCEGSFNGSEKETMQFLNDRLASYLEKVRQLERENAELESRIRERCQQQEPYVCPSYQSYFRTIEELQQKILCAKSENARLVVQIDNAKLAADDFRTKYETELGLRQLVESDINGLRRILDELTLCKSDLEAQVESLKEELLCLKRNHEEEVNTLRCQIGDRLNVEVDAAPAVDLNRVLNETRCQYEALVETNRRDVEEWFTTQTEELNKQVVSSSEQLQSCQAEIIELRRTVNALEIELQAQHNLRDSLENTLTETEARYSSQLSQLQCMITNVESQLAEIRSDLERQNQEYQVLLDVRARLECEINTYRGLLESEDCKLPCNPCATTNACGSSGSCVSNSCAPCTPCVPRPRCGPCNSFVRSGGSGGGHHHHHHGGSGGSHHHHHHDGGSGGGSTSRDHMVLHEYVNAAGIT

SEQ ID NO: 32 - protein, 538 aa, synthetic construct
  source 1..538: note = Gma UPO SP-KRT32-His2 fusion protein
MRGTPIFASLIALFAHAAIAFPAYGSLAGLTREQLDEILPTLEIRATSNCSASIKSCPRPSSVCSSSMSCRPEMCLGYVCQPVSCVPSVSMPTTYRPASCFSKTYLSSSCWAASGISSSMGTCSWFCEGSFNGNEKETMQSLNDRLACYLEKVRQLERENAELESKIQEACQSQVATMSPDYQSYFRTIEELQQKVLCTKAENARMVVHIDNAKLAADDFRTKYETELTMRQLVEADTNGLRRILDELTLCKADLEAQVESLKEELLCLKKNHEQEVSALRCQLGDRLNIEVDAAPPVDLNRMLEEMRCQYETVVEANLRDVEEWFNTQMEELNQQVATSSEQLQSYQSDIIDLRRTVNTLEIELQAQHSLRDSLESTLAETEARYGSQLAQMQCLISNVEAQLAEIRCDLERQNQEYKVLLDVKARLECEINTYRGLLESEDCKLPCNPCSTPSCPPCAPSPSMPRTVCVPRTVCVPCVPCPQSRFSGGSGGGHHHHHHGGSGGSHHHHHHDGGSGGGSTSRDHMVLHEYVNAAGIT

SEQ ID NO: 33 - protein, 652 aa, synthetic construct
  source 1..652: note = preostalpha SP-KRT82-His2 fusion protein
MRQVWFSWIVGLFLCFFNVSSAAPVNTTTEDETAQIPAEAVIGYSDLEGDFDVAVLPFSNSTNNGLLFINTTIASIAAKEEGVSLEKREAEASCRSFQLGSRCGGRSFSSCSAVLPRMVTHYAVSKGPCQSGGGSALRALGCLGSRSLCNVGFGRPRVASRCGLPGFGYRVGAPCGSSPCIAPVTINESLLVPLELEIDPAVQKVKRDEKEQIKCLNNRFASFINKVRFLEQKNKLLETKWNFMQQQRCCQSNIEPIFQAYISALRRQLDCVAGDRARLESELCSLQDVLESYKKKYEEELSLRPCAENEFVALKKDVDTAFLMKADLETNAEALVQEIDFLKGLYEEEICLLQSQISETSVIVKMDNSRELDVDGIIAEIKAQYDDIASRSKAEAEAWYQSRYEELRLTAGNHCDNLRNRKNEILEMNKLIQRLQQEIENVKAQRCKLEAAVTQAEQQGEAALSDAKCKLVGLEEALQKAKQDMACLLKEYQEVMNSKLGLDIEIATYRRLLEGEEHRLCEGIGPVNISVSSSKGAVLYEPCVVSTPVLRTGVLKTSGACSVVGTGEVYVPCEPQGLLSCVSTRSSCMKLGAGSSSSHKCSGGSGGGHHHHHHGGSGGSHHHHHHDGGSGGGSTSRDHMVLHEYVNAAGIT

SEQ ID NO: 34 - protein, 583 aa, synthetic construct
  source 1..583: note = Killer protein SP-KRT85-His2 fusion protein
MTKPTQVLVRSVSILFFITLLHLVVASCRSYRISSGCGVTRTFSSCSAVAPKTGNRCCISAAPYRGVSCYRGLTGFGSRSLSNLGSCGPRMAMGGFRAGSCGRSFGYRSGGVCGPSPPCITTVSVNESLLTPLNLEIDPNAQCVKHEEKEQIKCLNNRFAAFIDKVRFLEQQNKLLETKWQFYQNQRCCESNMEPLFNGYIETLRREAECVEADSGRLASELNHVQEVLEGYKKKYEEEVALRATAENEFVVLKKDVDCAYLRKSDLEANVEALVEESSFLKRLYDEELQVLHAHISDTSVIVKMDNSRDLNMDCVVAEIKAQYDDIASRSRAEAESWYRSKCEEMKATVIRHGETLRRTKEEINELNRMIQRLTAEIENAKCQRAKLEAAVAEAEQQGEAALTDARCKLAELEAALQKAKQDMACLLKEYQEVMNSKLGLDIEIATYRRLLEGEEHRLCEGVGSVNVCVSSSRGGVACGGLTCSTTPGRQIASGPVATGGSITVMAPDSCAPCQPRSSSFSCGSSRSVRFASGGSGGGHHHHHHGGSGGSHHHHHHDGGSGGGSTSRDHMVLHEYVNAAGIT

SEQ ID NO: 35 - protein, 531 aa, synthetic construct
  source 1..531: note = Killer protein SP-KRT35-His2 fusion protein
MTKPTQVLVRSVSILFFITLLHLVVAASKCLKASFSSGSLRGLGGAGGGSARVSAIYPSSSCKLPSLSRGARSFSACSVGLGRSSSRAAGCLSALCLPAGGFTTSYNLGGGWFGDGILTGSEKETMQSLNDRLASYLEKVRQLERENASLEGRIREWCEQQVPYLSPDYQSYFRTIEELQKKTLCTKAENARLVVQIDNAKLAADDFRTKYETELSMRQLVESDMNGLRRILDDLTLCKSDLEAQVESLKEELLCLKKNHEEEVNSLRCQLGDRLNVEVDAAPPVDLNRVLDEMRCQYETLVENNRRDAEEWFNTQTEELNQQVVSSSEQLQSCQAEIIELRRSVNALEIELQAQQSMRDALESTLAETEARYSSQLAQMQCLISNVEAQLAEIRSDLERQNQEYQVLLDVRARLECEINTYRGLLESEEGKLPCNPCAPDHTPGKSCLPCLPAVSCGPGAVRSTCSPRTICVPCPGGRFSGGSGGGHHHHHHGGSGGSHHHHHHDGGSGGGSTSRDHMVLHEYVNAAGIT

SEQ ID NO: 36 - protein, 656 aa, synthetic construct
  source 1..656: note = alpha factor SP-KRT81-His2 fusion protein
MRFPSIFTAVLFAASSALAAPVNTTTEDETAQIPAEAVIGYLDLEGDFDVAVLPFSNSTNNGLLFINTTIASIAAKEEGVSLDKREATCGSGFCGRAFSCISACGPRPGRCCITAAPYRGVSCYRGLTGGFGSHSVCGGFRAGSCGRSFGYRSGGVCGPSPPCITSVSVNESLLTPLNLEIDPNAQCVKHEEKEQIKCLNSRFAAFIDKVRFLEQQNKLLETKWQFYQNRKCCESNLEPLFEGYIETLRREAECVEADSGRLASELNHVQEVLEGYKKKYEEEVALRATAENEFVALKKDVDCAYLRKSDLEANAEALTEEIDFLRRLYEEEIRVLHAHISDTSVIVKMDNSRDLNMDCIVAEIKAQYDDIASRSRAEAESWYRSKCEEMKATVIRHGETLRRTKEEINELNRMIQRLTAEVENAKCQNTKLEAAVTQAEQQGETALSDARCKLAELEAALQKAKQDMACLVKEYQEVMNSKLGLDIEIATYRRLLEGEEQRLCEGVGAVNVCVSSSRGGVVCGDLCVSGSRPVTGSACSAPCSGNLAVSTGMCAPCAPCAPCAPCAPCGPCNSVTSCGLGTGGVGSCGISSCGVGSCASSCRRCSGGSGGGHHHHHHGGSGGSHHHHHHDGGSGGGSTSRDHMVLHEYVNAAGIT

SEQ ID NO: 37 - protein, 478 aa, synthetic construct
  source 1..478: note = 0030 SP-KRT31-His2 fusion protein
MKFAISTLLILQAAAVFAAPYNCCLPNVSCRSTCSSRPCVPPSCHTCTLPGACNIPANVGNCGWFCEGSFNGSEKETMQFLNDRLASYLEKVRQLERENAELESRIRERCQQQEPYVCPSYQSYFRTIEELQQKILCAKSENARLVVQIDNAKLAADDFRTKYETELGLRQLVESDINGLRRILDELTLCKSDLEAQVESLKEELLCLKRNHEEEVNTLRCQIGDRLNVEVDAAPAVDLNRVLNETRCQYEALVETNRRDVEEWFTTQTEELNKQVVSSSEQLQSCQAEIIELRRTVNALEIELQAQHNLRDSLENTLTETEARYSSQLSQLQCMITNVESQLAEIRSDLERQNQEYQVLLDVRARLECEINTYRGLLESEDCKLPCNPCATTNACGSSGSCVSNSCAPCTPCVPRPRCGPCNSFVRSGGSGGGHHHHHHGGSGGSHHHHHHDGGSGGGSTSRDHMVLHEYVNAAGIT

SEQ ID NO: 38 - protein, 511 aa, synthetic construct
  source 1..511: note = 0030 SP-KRT32-His2 fusion protein
MKFAISTLLILQAAAVFAATSNCSASIKSCPRPSSVCSSSMSCRPEMCLGYVCQPVSCVPSVSMPTTYRPASCFSKTYLSSSCWAASGISSSMGTCSWFCEGSFNGNEKETMQSLNDRLACYLEKVRQLERENAELESKIQEACQSQVATMSPDYQSYFRTIEELQQKVLCTKAENARMVVHIDNAKLAADDFRTKYETELTMRQLVEADTNGLRRILDELTLCKADLEAQVESLKEELLCLKKNHEQEVSALRCQLGDRLNIEVDAAPPVDLNRMLEEMRCQYETVVEANLRDVEEWFNTQMEELNQQVATSSEQLQSYQSDIIDLRRTVNTLEIELQAQHSLRDSLESTLAETEARYGSQLAQMQCLISNVEAQLAEIRCDLERQNQEYKVLLDVKARLECEINTYRGLLESEDCKLPCNPCSTPSCPPCAPSPSMPRTVCVPRTVCVPCVPCPQSRFSGGSGGGHHHHHHGGSGGSHHHHHHDGGSGGGSTSRDHMVLHEYVNAAGIT

SEQ ID NO: 39 - protein, 579 aa, synthetic construct
  source 1..579: note = 0030 SP-KRT82-His2 fusion protein
MKFAISTLLILQAAAVFAASCRSFQLGSRCGGRSFSSCSAVLPRMVTHYAVSKGPCQSGGGSALRALGCLGSRSLCNVGFGRPRVASRCGLPGFGYRVGAPCGSSPCIAPVTINESLLVPLELEIDPAVQKVKRDEKEQIKCLNNRFASFINKVRFLEQKNKLLETKWNFMQQQRCCQSNIEPIFQAYISALRRQLDCVAGDRARLESELCSLQDVLESYKKKYEEELSLRPCAENEFVALKKDVDTAFLMKADLETNAEALVQEIDFLKGLYEEEICLLQSQISETSVIVKMDNSRELDVDGIIAEIKAQYDDIASRSKAEAEAWYQSRYEELRLTAGNHCDNLRNRKNEILEMNKLIQRLQQEIENVKAQRCKLEAAVTQAEQQGEAALSDAKCKLVGLEEALQKAKQDMACLLKEYQEVMNSKLGLDIEIATYRRLLEGEEHRLCEGIGPVNISVSSSKGAVLYEPCVVSTPVLRTGVLKTSGACSVVGTGEVYVPCEPQGLLSCVSTRSSCMKLGAGSSSSHKCSGGSGGGHHHHHHGGSGGSHHHHHHDGGSGGGSTSRDHMVLHEYVNAAGIT

SEQ ID NO: 40 - protein, 576 aa, synthetic construct
  source 1..576: note = Invertase 2 SP-KRT85-His2 fusion protein
MLLQAFLFLLAGFAAKISASCRSYRISSGCGVTRTFSSCSAVAPKTGNRCCISAAPYRGVSCYRGLTGFGSRSLSNLGSCGPRMAMGGFRAGSCGRSFGYRSGGVCGPSPPCITTVSVNESLLTPLNLEIDPNAQCVKHEEKEQIKCLNNRFAAFIDKVRFLEQQNKLLETKWQFYQNQRCCESNMEPLFNGYIETLRREAECVEADSGRLASELNHVQEVLEGYKKKYEEEVALRATAENEFVVLKKDVDCAYLRKSDLEANVEALVEESSFLKRLYDEELQVLHAHISDTSVIVKMDNSRDLNMDCVVAEIKAQYDDIASRSRAEAESWYRSKCEEMKATVIRHGETLRRTKEEINELNRMIQRLTAEIENAKCQRAKLEAAVAEAEQQGEAALTDARCKLAELEAALQKAKQDMACLLKEYQEVMNSKLGLDIEIATYRRLLEGEEHRLCEGVGSVNVCVSSSRGGVACGGLTCSTTPGRQIASGPVATGGSITVMAPDSCAPCQPRSSSFSCGSSRSVRFASGGSGGGHHHHHHGGSGGSHHHHHHDGGSGGGSTSRDHMVLHEYVNAAGIT

SEQ ID NO: 41 - protein, 510 aa, synthetic construct
  source 1..510: note = Mink KRT 82 N437A mutant protein
MSCRSFQLGSRCGGRSFSSCSAVLPRMVTHYAVSKGPCQSGGGSALRALGCLGSRSLCNVGFGRPRVASRCGLPGFGYRVGAPCGSSPCIAPVTINESLLVPLELEIDPAVQKVKRDEKEQIKCLNNRFASFINKVRFLEQKNKLLETKWNFMQQQRCCQSNIEPIFQAYISALRRQLDCVAGDRARLESELCSLQDVLESYKKKYEEELSLRPCAENEFVALKKDVDTAFLMKADLETNAEALVQEIDFLKGLYEEEICLLQSQISETSVIVKMDNSRELDVDGIIAEIKAQYDDIASRSKAEAEAWYQSRYEELRLTAGNHCDNLRNRKNEILEMNKLIQRLQQEIENVKAQRCKLEAAVTQAEQQGEAALSDAKCKLVGLEEALQKAKQDMACLLKEYQEVMNSKLGLDIEIATYRRLLEGEEHRLCEGIGPVAISVSSSKGAVLYEPCVVSTPVLRTGVLKTSGACSVVGTGEVYVPCEPQGLLSCVSTRSSCMKLGAGSSSSHKC

SEQ ID NO: 42 - protein, 510 aa, synthetic construct
  source 1..510: note = Mink KRT 82 N437E mutant protein
MSCRSFQLGSRCGGRSFSSCSAVLPRMVTHYAVSKGPCQSGGGSALRALGCLGSRSLCNVGFGRPRVASRCGLPGFGYRVGAPCGSSPCIAPVTINESLLVPLELEIDPAVQKVKRDEKEQIKCLNNRFASFINKVRFLEQKNKLLETKWNFMQQQRCCQSNIEPIFQAYISALRRQLDCVAGDRARLESELCSLQDVLESYKKKYEEELSLRPCAENEFVALKKDVDTAFLMKADLETNAEALVQEIDFLKGLYEEEICLLQSQISETSVIVKMDNSRELDVDGIIAEIKAQYDDIASRSKAEAEAWYQSRYEELRLTAGNHCDNLRNRKNEILEMNKLIQRLQQEIENVKAQRCKLEAAVTQAEQQGEAALSDAKCKLVGLEEALQKAKQDMACLLKEYQEVMNSKLGLDIEIATYRRLLEGEEHRLCEGIGPVEISVSSSKGAVLYEPCVVSTPVLRTGVLKTSGACSVVGTGEVYVPCEPQGLLSCVSTRSSCMKLGAGSSSSHKC

SEQ ID NO: 43 - protein, 652 aa, synthetic construct
  source 1..652: note = preostalpha SP-KRT82_N437A-His2 fusion protein
MRQVWFSWIVGLFLCFFNVSSAAPVNTTTEDETAQIPAEAVIGYSDLEGDFDVAVLPFSNSTNNGLLFINTTIASIAAKEEGVSLEKREAEASCRSFQLGSRCGGRSFSSCSAVLPRMVTHYAVSKGPCQSGGGSALRALGCLGSRSLCNVGFGRPRVASRCGLPGFGYRVGAPCGSSPCIAPVTINESLLVPLELEIDPAVQKVKRDEKEQIKCLNNRFASFINKVRFLEQKNKLLETKWNFMQQQRCCQSNIEPIFQAYISALRRQLDCVAGDRARLESELCSLQDVLESYKKKYEEELSLRPCAENEFVALKKDVDTAFLMKADLETNAEALVQEIDFLKGLYEEEICLLQSQISETSVIVKMDNSRELDVDGIIAEIKAQYDDIASRSKAEAEAWYQSRYEELRLTAGNHCDNLRNRKNEILEMNKLIQRLQQEIENVKAQRCKLEAAVTQAEQQGEAALSDAKCKLVGLEEALQKAKQDMACLLKEYQEVMNSKLGLDIEIATYRRLLEGEEHRLCEGIGPVAISVSSSKGAVLYEPCVVSTPVLRTGVLKTSGACSVVGTGEVYVPCEPQGLLSCVSTRSSCMKLGAGSSSSHKCSGGSGGGHHHHHHGGSGGSHHHHHHDGGSGGGSTSRDHMVLHEYVNAAGIT

SEQ ID NO: 44 - protein, 652 aa, synthetic construct
  source 1..652: note = preostalpha SP-KRT82_N437E-His2 fusion protein
MRQVWFSWIVGLFLCFFNVSSAAPVNTTTEDETAQIPAEAVIGYSDLEGDFDVAVLPFSNSTNNGLLFINTTIASIAAKEEGVSLEKREAEASCRSFQLGSRCGGRSFSSCSAVLPRMVTHYAVSKGPCQSGGGSALRALGCLGSRSLCNVGFGRPRVASRCGLPGFGYRVGAPCGSSPCIAPVTINESLLVPLELEIDPAVQKVKRDEKEQIKCLNNRFASFINKVRFLEQKNKLLETKWNFMQQQRCCQSNIEPIFQAYISALRRQLDCVAGDRARLESELCSLQDVLESYKKKYEEELSLRPCAENEFVALKKDVDTAFLMKADLETNAEALVQEIDFLKGLYEEEICLLQSQISETSVIVKMDNSRELDVDGIIAEIKAQYDDIASRSKAEAEAWYQSRYEELRLTAGNHCDNLRNRKNEILEMNKLIQRLQQEIENVKAQRCKLEAAVTQAEQQGEAALSDAKCKLVGLEEALQKAKQDMACLLKEYQEVMNSKLGLDIEIATYRRLLEGEEHRLCEGIGPVEISVSSSKGAVLYEPCVVSTPVLRTGVLKTSGACSVVGTGEVYVPCEPQGLLSCVSTRSSCMKLGAGSSSSHKCSGGSGGGHHHHHHGGSGGSHHHHHHDGGSGGGSTSRDHMVLHEYVNAAGIT